European Patent Specification EP 4 069 849 B1, published January 22, 2025. Title: LIVER-SPECIFIC PROMOTER AND APPLICATION THEREOF. The sequence listing filed with the application follows.

SEQUENCE LISTING (10 sequences)

SEQ ID NO: 1 - DNA, 204 bp, Human
tgtctgtctgcacatttcgtagagcgagtgttccgatactctaatctccctaggcaaggttcatatttgtgtaggttacttattctccttttgttgactaagtcaataatcagaatcagcaggtttggagtcagcttggcagggatcagcagcctgggttggaaggagggggtataaaagccccttcaccaggagaagccgtca

SEQ ID NO: 2 - DNA, 152 bp, Human
ggcaaggttcatatttgtgtaggttacttattctccttttgttgactaagtcaataatcagaatcagcaggtttggagtcagcttggcagggatcagcagcctgggttggaaggagggggtataaaagccccttcaccaggagaagccgtca

SEQ ID NO: 3 - DNA, 81 bp, Human
gggcgactcagatcccagccagtggacttagcccctgtttgctcctccgataactggggtgaccttggttaatattcacca

SEQ ID NO: 4 - DNA, 54 bp, Human
ccaccccctccaccttggacacaggacgctgtggtttctgagccaggtacaatg

SEQ ID NO: 5 - DNA, 99 bp, Human
tacctgctgatcgcccggcccctgttcaaacatgtcctaatactctgtctctgcaagggtcatcagtagttttccatcttactcaacatcctcccagtg

SEQ ID NO: 6 - DNA, 232 bp, Artificial Sequence
gggcgactcagatcccagccagtggacttagcccctgtttgctcctccgataactggggtgaccttggttaatattcaccaggcaaggttcatatttgtgtaggttacttattctccttttgttgactaagtcaataatcagaatcagcaggtttggagtcagcttggcagggatcagcagcctgggttggaaggagggggtataaaagccccttcaccaggagaagccgtc

SEQ ID NO: 7 - DNA, 284 bp, Artificial Sequence
gggcgactcagatcccagccagtggacttagcccctgtttgctcctccgataactggggtgaccttggttaatattcaccatgtctgtctgcacatttcgtagagcgagtgttccgatactctaatctccctaggcaaggttcatatttgtgtaggttacttattctccttttgttgactaagtcaataatcagaatcagcaggtttggagtcagcttggcagggatcagcagcctgggttggaaggagggggtataaaagccccttcaccaggagaagccgtc

SEQ ID NO: 8 - DNA, 287 bp, Artificial Sequence
ccaccccctccaccttggacacaggacgctgtggtttctgagccaggtacaatggggcgactcagatcccagccagtggacttagcccctgtttgctcctccgataactggggtgaccttggttaatattcaccaggcaaggttcatatttgtgtaggttacttattctccttttgttgactaagtcaataatcagaatcagcaggtttggagtcagcttggcagggatcagcagcctgggttggaaggagggggtataaaagccccttcaccaggagaagccgtca

SEQ ID NO: 9 - DNA, 338 bp, Artificial Sequence
ccaccccctccaccttggacacaggacgctgtggtttctgagccaggtacaatggggcgactcagatcccagccagtggacttagcccctgtttgctcctccgataactggggtgaccttggttaatattcaccatgtctgtctgcacatttcgtagagcgagtgttccgatactctaatctccctaggcaaggttcatatttgtgtaggttacttattctccttttgttgactaagtcaataatcagaatcagcaggtttggagtcagcttggcagggatcagcagcctgggttggaaggagggggtataaaagccccttcaccaggagaagccgtc

SEQ ID NO: 10 - DNA, 331 bp, Artificial Sequence
tacctgctgatcgcccggcccctgttcaaacatgtcctaatactctgtctctgcaagggtcatcagtagttttccatcttactcaacatcctcccagtggggcgactcagatcccagccagtggacttagcccctgtttgctcctccgataactggggtgaccttggttaatattcaccaggcaaggttcatatttgtgtaggttacttattctccttttgttgactaagtcaataatcagaatcagcaggtttggagtcagcttggcagggatcagcagcctgggttggaaggagggggtataaaagccccttcaccaggagaagccgtc